European Patent Application EP 4 541 816 A1, published April 23, 2025. Title: ANTI-CLDN18.2 ANTIBODY, AND PHARMACEUTICAL COMPOSITION AND USE THEREOF. Applicant: AKESO BIOPHARMA, INC. Application WO PCT/CN2023/100225, filed June 14, 2023. The sequence listing filed with the application follows.

SEQUENCE LISTING (26 sequences)

SEQ ID NO: 1 - DNA, 354 bp, synthetic construct
  source 1..354: mol_type = other DNA; note = nucleic acid sequence encoding 8C5.1VH
gaagtgcagctggttgagagcggcggaggactggtgaaacctggaggatctctgaagctgagctgcgctgcttccggattcacttttagcaactccgccgtgagctgggtgagacaaacacctgagaagaggctggagtgggtggctacaatcacaagcggcgtgagctacacctactacctggactccgtgaggggcagattcacaatcagcagggacaacgccaagaacaccctgtacctgcagatgagcagcctgaggagcgaggataccgctatgtactactgtaccaggcagttcaagggcaacgccctggattactggggccaaggaacctctgtgacagtgagctcc

SEQ ID NO: 2 - protein, 118 aa, synthetic construct
  source 1..118: note = 8C5.1VH
EVQLVESGGGLVKPGGSLKLSCAASGFTFSNSAVSWVRQTPEKRLEWVATITSGVSYTYYLDSVRGRFTISRDNAKNTLYLQMSSLRSEDTAMYYCTRQFKGNALDYWGQGTSVTVSS

SEQ ID NO: 3 - DNA, 339 bp, synthetic construct
  source 1..339: mol_type = other DNA; note = nucleic acid sequence encoding 8C5.1VL
gacattgtgatgacccagtccccttcctccctgacagtgacagctggagagaaggtgacaatgtcctgcaagagcagccagagcctgctgaactccggaaatcagaagaactacctgacctggtaccagcagaagcccggacaaccacctaagctgctgatctactgggcctccaccagggaaagcggagttcctgatagattcaccggcagcggctccggaacagatttcacactgacaatcaacaacttccaggctgaggacctggccgtgtactactgtcagaacgactacttctaccctctgaccttcggcgccggaacaaagctggaactgaag

SEQ ID NO: 4 - protein, 113 aa, synthetic construct
  source 1..113: note = 8C5.1VL
DIVMTQSPSSLTVTAGEKVTMSCKSSQSLLNSGNQKNYLTWYQQKPGQPPKLLIYWASTRESGVPDRFTGSGSGTDFTLTINNFQAEDLAVYYCQNDYFYPLTFGAGTKLELK

SEQ ID NO: 5 - protein, 8 aa, synthetic construct
  source 1..8: note = 8C5.1 HCDR1
GFTFSNSA

SEQ ID NO: 6 - protein, 8 aa, synthetic construct
  source 1..8: note = 8C5.1 HCDR2
ITSGVSYT

SEQ ID NO: 7 - protein, 11 aa, synthetic construct
  source 1..11: note = 8C5.1 HCDR3
TRQFKGNALDY

SEQ ID NO: 8 - protein, 12 aa, synthetic construct
  source 1..12: note = 8C5.1 LCDR1
QSLLNSGNQKNY

SEQ ID NO: 9 - skipped

SEQ ID NO: 10 - protein, 9 aa, synthetic construct
  source 1..9: note = 8C5.1 LCDR3
QNDYFYPLT

SEQ ID NO: 11 - protein, 118 aa, synthetic construct
  source 1..118: note = 8C5.1 H1VH
EVQLVESGGGLVKPGGSLRLSCAASGFTFSNSAVSWVRQAPGKRLEWVATITSGVSYTYYLDSVRGRFTISRDNAKNSLYLQMNSLRAEDTAVYYCTRQFKGNALDYWGQGTSVTVSS

SEQ ID NO: 12 - DNA, 354 bp, synthetic construct
  source 1..354: mol_type = other DNA; note = nucleic acid sequence encoding 8C5.1 H1VH
gaggtgcagctggtggagagcggcggcggcctggtgaagcccggcggcagcctgaggctgtcctgcgccgcctctggcttcaccttttctaacagcgccgtgtcttgggtgaggcaggcacctggcaagcgcctggagtgggtggccaccatcacatccggcgtgtcttacacctactatctggacagcgtgcggggcagattcacaatcagcagagataacgccaagaacagcctgtatctgcagatgaactctctgcgggccgaggacaccgccgtgtactattgtacaagacagtttaagggcaatgccctggattactggggccagggcaccagcgtgacagtgagctcc

SEQ ID NO: 13 - protein, 118 aa, synthetic construct
  source 1..118: note = 8C5.1 H2VH
EVQLVESGGGLVKPGGSLRLSCAASGFTFSNSAVSWVRQAPGKGLEWVSTITSGVSYTYYADSVKGRFTISRDNAKNSLYLQMNSLRAEDTAVYYCTRQFKGNALDYWGQGTSVTVSS

SEQ ID NO: 14 - DNA, 354 bp, synthetic construct
  source 1..354: mol_type = other DNA; note = nucleic acid sequence encoding 8C5.1 H2VH
gaggtgcagctggtggagagcggcggcggcctggtgaagcccggcggcagcctgaggctgtcctgcgcagcatctggcttcaccttttctaacagcgccgtgtcttgggtgaggcaggcacctggcaagggactggagtgggtgagcaccatcacatccggcgtgtcttacacctactatgccgactccgtgaagggccggttcacaatcagcagagataacgccaagaacagcctgtatctgcagatgaactctctgagggccgaggacaccgccgtgtactattgtacacgccagtttaagggcaatgccctggattactggggccagggcaccagcgtgacagtgagctcc

SEQ ID NO: 15 - protein, 118 aa, synthetic construct
  source 1..118: note = 8C5.1 H3VH
EVQLVESGGGLVKPGGSLRLSCAASGFTFSNSAVSWVRQAPGKGLEWVSSITSGVSYTYYADSVKGRFTISRDNAKNSLYLQMNSLRAEDTAVYYCTRQFKGNALDYWGQGTSVTVSS

SEQ ID NO: 16 - DNA, 354 bp, synthetic construct
  source 1..354: mol_type = other DNA; note = nucleic acid sequence encoding 8C5.1 H3VH
gaggtgcagctggtggagagcggcggcggcctggtgaagcccggcggcagcctgaggctgtcctgcgcagcatctggcttcaccttttctaacagcgccgtgtcttgggtgaggcaggcacctggcaagggactggagtgggtgagctccatcacatccggcgtgtcttacacctactatgccgactccgtgaagggccggttcacaatcagcagagataacgccaagaacagcctgtatctgcagatgaactctctgagggccgaggacaccgccgtgtactattgtacacgccagtttaagggcaatgccctggattactggggccagggcaccagcgtgacagtgagctcc

SEQ ID NO: 17 - protein, 113 aa, synthetic construct
  source 1..113: note = 8C5.1 L1VL
DIVMTQSPSSLSVSPGERVTMSCKSSQSLLNSGNQKNYLTWYQQKPGQPPKLLIYWASTRESGVPDRFSGSGSGTDFTLTINSFQAEDVAVYYCQNDYFYPLTFGAGTKLELK

SEQ ID NO: 18 - DNA, 339 bp, synthetic construct
  source 1..339: mol_type = other DNA; note = nucleic acid sequence encoding 8C5.1 L1VL
gatatcgtgatgacccagagcccatctagcctgtccgtgtctccaggcgagagagtgaccatgagctgcaagtcttcccagagcctgctgaatagcggcaaccagaagaactacctgacatggtaccagcagaagccaggccagcctccaaagctgctgatctactgggccagcacaagagagagcggcgtgccagacagattctctggcagcggctctggcaccgacttcacactgaccatcaactccttccaggccgaggatgtggccgtgtattactgccagaacgattacttctatcccctgacattcggcgccggcacaaagctggagctgaag

SEQ ID NO: 19 - protein, 113 aa, synthetic construct
  source 1..113: note = 8C5.1 L2VL
DIVMTQSPSSLSVSPGERVTISCKSSQSLLNSGNQKNYLTWYQQKPGQPPKLLIYWASTRESGVPDRFSGSGSGTDFTLTISSFQAEDVAVYYCQNDYFYPLTFGAGTKLELK

SEQ ID NO: 20 - DNA, 339 bp, synthetic construct
  source 1..339: mol_type = other DNA; note = nucleic acid sequence encoding 8C5.1 L2VL
gacatcgtgatgacccagtctccaagctccctgagcgtgtccccaggagagagggtgacaatctcctgcaagtctagccagtctctgctgaacagcggcaatcagaagaactacctgacctggtatcagcagaagcctggccagccccctaagctgctgatctactgggcctccaccagggagtctggagtgccagacagattttctggcagcggctccggcacagatttcaccctgacaatctcctcttttcaggccgaggacgtggccgtgtactattgtcagaatgattacttctatcccctgacctttggcgccggcacaaagctggagctgaag

SEQ ID NO: 21 - protein, 113 aa, synthetic construct
  source 1..113: note = 8C5.1 L3VL
DIVMTQSPSSLSVSPGERVTISCKSSQSLLNSGNQKNYLAWYQQKPGQPPKLLIYWASTRESGVPDRFSGSGSGTDFTLTISSLQAEDVAVYYCQNDYFYPLTFGAGTKLELK

SEQ ID NO: 22 - DNA, 339 bp, synthetic construct
  source 1..339: mol_type = other DNA; note = nucleic acid sequence encoding 8C5.1 L3VL
gacatcgtgatgacccagtctccaagctccctgagcgtgtccccaggagagagggtgacaatctcctgcaagtctagccagtctctgctgaacagcggcaatcagaagaactacctggcctggtatcagcagaagcctggccagccccctaagctgctgatctactgggcctccaccagggagtctggagtgccagacagattctctggcagcggctccggcacagacttcaccctgacaatctcctctctgcaggccgaggacgtggccgtgtactattgtcagaatgattacttctatcccctgacctttggcgccggcacaaagctggagctgaag

SEQ ID NO: 23 - protein, 330 aa, synthetic construct
  source 1..330: note = Amino acid sequence of the heavy chain constant region of hG1WT
ASTKGPSVFPLAPSSKSTSGGTAALGCLVKDYFPEPVTVSWNSGALTSGVHTFPAVLQSSGLYSLSSVVTVPSSSLGTQTYICNVNHKPSNTKVDKKVEPKSCDKTHTCPPCPAPELLGGPSVFLFPPKPKDTLMISRTPEVTCVVVDVSHEDPEVKFNWYVDGVEVHNAKTKPREEQYNSTYRVVSVLTVLHQDWLNGKEYKCKVSNKALPAPIEKTISKAKGQPREPQVYTLPPSREEMTKNQVSLTCLVKGFYPSDIAVEWESNGQPENNYKTTPPVLDSDGSFFLYSKLTVDKSRWQQGNVFSCSVMHEALHNHYTQKSLSLSPGK

SEQ ID NO: 24 - protein, 107 aa, synthetic construct [sequence omitted]

SEQ ID NO: 25 - protein, 448 aa, synthetic construct
  source 1..448: note = Amino acid sequence of heavy chain of positive control antibody IMAB362
QVQLQQPGAELVRPGASVKLSCKASGYTFTSYWINWVKQRPGQGLEWIGNIYPSDSYTNYNQKFKDKATLTVDKSSSTAYMQLSSPTSEDSAVYYCTRSWRGNSFDYWGQGTTLTVSSASTKGPSVFPLAPSSKSTSGGTAALGCLVKDYFPEPVTVSWNSGALTSGVHTFPAVLQSSGLYSLSSVVTVPSSSLGTQTYICNVNHKPSNTKVDKRVEPKSCDKTHTCPPCPAPELLGGPSVFLFPPKPKDTLMISRTPEVTCVVVDVSHEDPEVKFNWYVDGVEVHNAKTKPREEQYNSTYRVVSVLTVLHQDWLNGKEYKCKVSNKALPAPIEKTISKAKGQPREPQVYTLPPSREEMTKNQVSLTCLVKGFYPSDIAVEWESNGQPENNYKTTPPVLDSDGSFFLYSKLTVDKSRWQQGNVFSCSVMHEALHNHYTQKSLSLSPGK

SEQ ID NO: 26 - protein, 220 aa, synthetic construct
  source 1..220: note = Amino acid sequence of light chain of positive control antibody IMAB362
DIVMTQSPSSLTVTAGEKVTMSCKSSQSLLNSGNQKNYLTWYQQKPGQPPKLLIYWASTRESGVPDRFTGSGSGTDFTLTISSVQAEDLAVYYCQNDYSYPFTFGSGTKLEIKRTVAAPSVFIFPPSDEQLKSGTASVVCLLNNFYPREAKVQWKVDNALQSGNSQESVTEQDSKDSTYSLSSTLTLSKADYEKHKVYACEVTHQGLSSPVTKSFNRGEC